European Patent Application EP 4 628 096 A1, published October 8, 2025. Title: 구제역 바이러스 유사 입자 또는 나노입자 생산을 위한 재조합 발현 벡터 및 이를 이용한 백신 조성물. Applicant: Optipharm.CO.,LTD. The sequence listing filed with the application follows.

SEQUENCE LISTING (24 sequences)

SEQ ID NO: 1 - DNA, 633 bp, Foot-and-mouth disease virus
  source 1..633: mol_type = other DNA
accacatcgacaggagagtcggctgaccccgtgactgccaccgtagaaaattatggcggcgagacacaggtgcagaggcgccatcacacagacgtttcattcatactagacagatttgtgaaagtcactccaaaagactcaataaatgtcttggacctgatgcagaccccctcccataccctagtaggagcgctacttcgcactgctacttactatttcgctgatttagaggtggctgtgaaacatgagggagaccttacctgggttccaaatggagcacctgaagcggccttggataataccaccaacccaacggcgtaccataaggcgccgttgactcggctcgcattgccatatacggcaccacatcgtgttttagccaccgtgtacaatgggaactgcaagtacgctggtggatcactgcccaacgtgagaggcgacctccaagtgctggctcagaaggcagcgcgtccactacctacttctttcaactacggtgccattaaagccactcgcgtgacagaactgctgtaccgcatgaagagggccgaaacatactgtcctaggcccctcttagctgttcacccaagcgcggcccgacacaagcagaaaatagtagcccctgttaagcag

SEQ ID NO: 2 - DNA, 654 bp, Foot-and-mouth disease virus
  source 1..654: mol_type = other DNA
gataagaaaaccgaagagacgactctgctcgaggatcgtatcctcactacccgaaacggacacacaacctcgacaacccagtcgagtgttggtattactcacggttacgcaactgctgaagattttgttagtggcccaaacacctctggtcttgagactagagttgtccaagcggaaaggttcttcaaaacccacctgttcgactgggtaacatcggatcctttcggaaggtgctatttgttggaactcccgactgatcacaaaggtgtctacggctctctgaccgattcatacgcctacatgagaaacggttgggatgttgaagtcaccgctgtgggcaatcaattcaacggaggctgcctactggtggccatggtgcctgaattatgttctatcgatcggagagaactgttccagctgacgctcttcccccaccagttcatcaacccccgcacgaacatgacagcccacatcaaggtgccctttgttggcgtcaaccgttatgatcagtacaaggtacacaagccgtggaccctcgtagttatggtcgtagccccactgactgtaaacactgaaggcgctccgcagatcaaggtgtatgctaatatcgcaccaaccaacgtgcatgtagccggtgagttcccttccaaagag

SEQ ID NO: 3 - DNA, 660 bp, Foot-and-mouth disease virus
  source 1..660: mol_type = other DNA
gggattttccctgtggcctgtagcgacggttacggaggcttggtgacaactgacccaaagacagctgaccccgtctatggtaaagtgttcaacccccctcgcaacatgttgcctgggcgtttcaccaacctcctggacgtggctgaggcttgccccacgtttctgcacttcgatggtgacgtaccgtatgtgactactaagacggattcggacagggtgcttgcacaatttgatttgtctttggcagcaaagcacatgagcaacaccttccttgcaggtctggcccagtattacacgcaatacagcggcaccgtcaatctgcatttcatgttcacaggtcccacggatgcgaaggcgcgttacatgattgcgtatgcccctccaggcatggagccgcccaaaacaccagaagctgctgctcactgcattcacgcagagtgggacacgggtctgaactcaaagttcacattttccatcccctacctcagcgcggctgattacgcgtacaccgcgtctgacgctgctgagaccacgaatgttcagggatgggtctgcttattccaaattacacatgggaaggctgaaggtgacgctcttgtcgtgatggccagtgctggcaaggactttgagttgcgcctgcctgtggacgctcgtcaacag

SEQ ID NO: 4 - DNA, 255 bp, Foot-and-mouth disease virus
  source 1..255: mol_type = other DNA
ggagccggacaaagtagtccggctactggatcacagaaccaatcaggcaacaccggtagtatcatcaacaattactacatgcagcaataccagaactccatggacacacaacttggtgacaatgctatcagcggaggctccaacgagggatccacagacacaacttccacccacacaaccaacactcaaaacaatgactggttttcaaagttggccagctctgccttcagcggccttttcggcgctttgctcgcc

SEQ ID NO: 5 - DNA, 630 bp, Foot-and-mouth disease virus
  source 1..630: mol_type = other DNA
accaccgccaccggggaatcagcagaccctgtcacaaccaccgttgagaactacggtggcgagacacaagtacagcggcgttaccacaccgacgtcggcttcttaatggacaggttcgtgcagatcaagcctgagggccccacacatgtcattgacctcatgcagacacaccaacacgggctggtgggcgccatgttgcgcgcggccacctactacttttctgatcttgagattgtggtgaaccacacgggtaacctaacgtgggtacccaatggagcacccgaggcagcactgcaaaacacgagcaaccccactgcttaccacaaagcgccgttcacgaggcttgcgctcccctacaccgcgccacaccgcgtgctggcaactgtgtacagtgggacgagcaagtactccgcacctcaaaaccggcgaggtgacttgggtcctctcgcggcgagactcgctgcacaactccctgcctccttcaacttcggtgcaattcgggccacggagatccgcgaactccttgtgcgcatgaagcgcgccgagctctactgccccaggccactgttggcggtggaggtgtcgtcgcaagacagacacaagcagaaaatcattgcccctgcaaaacaa

SEQ ID NO: 6 - DNA, 654 bp, Foot-and-mouth disease virus
  source 1..654: mol_type = other DNA
gacaagaagaccgaagagacaactcttctggaggaccgtatcctcaccactcgtaatggacacaccacttctacaactcagtcgagtgtgggggtcacctacgggtattcaactggtgaggaccacgtttctggacctaacacatcaggtttggagacgcgggtggtacaagctgaaaggttcttcaagaagcacttgtttgattggacgacggacaaaccctttggtcacgttgaaaagctggaacttcccactgatcacaaaggtgtctacggacagctggtggactcctttgcatacatgagaaatggctgggacgtggaggtgtctgctgttggcaaccagttcaacggcgggtgccttctcgtggccatggtacctgagtttaaggagttcaccacacgtgaaaagtaccagctcaccctgttcccccaccagttcattagccccagaaccaacatgaccgcgcacatcacggtcccgtaccttggtgtgaacaggtatgaccagtacaacaaacacaaaccctggacgttggtggtgatggtggtttcaccacttaccactagctccattggtgcatcacagattaaggtctacaccaatatcgcccctacccacgttcacgtggctggcgagctcccgtcgaaagag

SEQ ID NO: 7 - DNA, 663 bp, Foot-and-mouth disease virus
  source 1..663: mol_type = other DNA
gggatcgtgccggtcgcctgctcggacgggtacggtggcctggtgacaacagaccctaaaacagctgaccctgcttacggtatggtgtacaacccacctaggaccaactaccccgggcggtttacaaacttgttggacgtggcagaggcgtgtcccaccttcctctgtttcgacgacgggaaaccgtatgttgtgacaagaacggatgagcagcgcctcttggccaagtttgacctttcccttgctgcaaagcacatgtcaaacacctacctttcagggatagcacagtactacgcacagtactctggcaccatcaatttgcacttcatgtttactggttccactgactcaaaggcccgttacatggtggcttacgtcccgcctggcgtgacaacgccaccggacacgcctgagagagctgcgcactgcatccacgcagaatgggacacggggctaaactccaaattcactttttcaatcccgtacgtatctgctgcagattacgcgtacacagcgtccgatgtggcagacacaacaaacgtacagggatgggtttgcatctaccaaatcacccacgggaaggccgaacaagacactttggtcgtgtcggtcagcgccggcaaagactttgagctgcgcctccccattgacccccgtgcgcaa

SEQ ID NO: 8 - DNA, 255 bp, Foot-and-mouth disease virus
  source 1..255: mol_type = other DNA
ggggcagggcaatctagccctgccaccgggtcacagaaccagtcaggcaataccggcagcattattaacaactactacatgcagcagtaccagaactccatggacacacaacttggtgacaacgccatcagcggaggatccaacgaggggtccacggacacaacctctacccacacaaccaacacccaaaacaatgactggttctcaaaactggcaagttccgcgttcaccggtcttttcggcgcactgctcgcc

SEQ ID NO: 9 - DNA, 642 bp, Foot-and-mouth disease virus
  source 1..642: mol_type = other DNA
agtggtgcccccccgaccgacttgcaaaagatggtcatgggtaataccaagcccgttgagctcatactcgacgggaagacagtagccatctgctgtgctactggagtatttggcactgcctacctcgtgcctcgtcatcttttcgctgagaagtacgacaagatcatgttggacggtagaaccatgacagacagtgactacagagtgtttgagtttgagattaaagtaaaaggacaggacatgctctcagacgctgcgctcatggtgctgcaccgtgggaaccgcgtgagagacatcacgaaacactttcgtgacacagcaagaatgaagaaaggcacccccatcgttggtgtgatcaacaacgctgacgtcgggagactgattttctcaggcgaggccctcacctacaaggacattgtagtgtgcatggatggagacaccatgccgggcctatttgcctataaagccgccaccaaggctggctactgcgggggagccgtccttgctaaggatggagccgacacattcatcgttggcactcactctgcaggtggcaacggagttgggtactgctcatgcgtatccagatccatgctccaaaaaatgaaggcacacatcgaccctgaaccacaccacgagtag

SEQ ID NO: 10 - protein, 211 aa, Foot-and-mouth disease virus
TTSTGESADPVTATVENYGGETQVQRRHHTDVSFILDRFVKVTPKDSINVLDLMQTPSHTLVGALLRTATYYFADLEVAVKHEGDLTWVPNGAPEAALDNTTNPTAYHKAPLTRLALPYTAPHRVLATVYNGNCKYAGGSLPNVRGDLQVLAQKAARPLPTSFNYGAIKATRVTELLYRMKRAETYCPRPLLAVHPSAARHKQKIVAPVKQ

SEQ ID NO: 11 - protein, 218 aa, Foot-and-mouth disease virus
DKKTEETTLLEDRILTTRNGHTTSTTQSSVGITHGYATAEDFVSGPNTSGLETRVVQAERFFKTHLFDWVTSDPFGRCYLLELPTDHKGVYGSLTDSYAYMRNGWDVEVTAVGNQFNGGCLLVAMVPELCSIDRRELFQLTLFPHQFINPRTNMTAHIKVPFVGVNRYDQYKVHKPWTLVVMVVAPLTVNTEGAPQIKVYANIAPTNVHVAGEFPSKE

SEQ ID NO: 12 - protein, 220 aa, Foot-and-mouth disease virus
GIFPVACSDGYGGLVTTDPKTADPVYGKVFNPPRNMLPGRFTNLLDVAEACPTFLHFDGDVPYVTTKTDSDRVLAQFDLSLAAKHMSNTFLAGLAQYYTQYSGTVNLHFMFTGPTDAKARYMIAYAPPGMEPPKTPEAAAHCIHAEWDTGLNSKFTFSIPYLSAADYAYTASDAAETTNVQGWVCLFQITHGKAEGDALVVMASAGKDFELRLPVDARQQ

SEQ ID NO: 13 - protein, 85 aa, Foot-and-mouth disease virus
GAGQSSPATGSQNQSGNTGSIINNYYMQQYQNSMDTQLGDNAISGGSNEGSTDTTSTHTTNTQNNDWFSKLASSAFSGLFGALLA

SEQ ID NO: 14 - protein, 210 aa, Foot-and-mouth disease virus
TTATGESADPVTTTVENYGGETQVQRRYHTDVGFLMDRFVQIKPEGPTHVIDLMQTHQHGLVGAMLRAATYYFSDLEIVVNHTGNLTWVPNGAPEAALQNTSNPTAYHKAPFTRLALPYTAPHRVLATVYSGTSKYSAPQNRRGDLGPLAARLAAQLPASFNFGAIRATEIRELLVRMKRAELYCPRPLLAVEVSSQDRHKQKIIAPAKQ

SEQ ID NO: 15 - protein, 218 aa, Foot-and-mouth disease virus
DKKTEETTLLEDRILTTRNGHTTSTTQSSVGVTYGYSTGEDHVSGPNTSGLETRVVQAERFFKKHLFDWTTDKPFGHVEKLELPTDHKGVYGQLVDSFAYMRNGWDVEVSAVGNQFNGGCLLVAMVPEFKEFTTREKYQLTLFPHQFISPRTNMTAHITVPYLGVNRYDQYNKHKPWTLVVMVVSPLTTSSIGASQIKVYTNIAPTHVHVAGELPSKE

SEQ ID NO: 16 - protein, 221 aa, Foot-and-mouth disease virus
GIVPVACSDGYGGLVTTDPKTADPAYGMVYNPPRTNYPGRFTNLLDVAEACPTFLCFDDGKPYVVTRTDEQRLLAKFDLSLAAKHMSNTYLSGIAQYYAQYSGTINLHFMFTGSTDSKARYMVAYVPPGVTTPPDTPERAAHCIHAEWDTGLNSKFTFSIPYVSAADYAYTASDVADTTNVQGWVCIYQITHGKAEQDTLVVSVSAGKDFELRLPIDPRAQ

SEQ ID NO: 17 - protein, 85 aa, Foot-and-mouth disease virus; identical to SEQ ID NO: 13

SEQ ID NO: 18 - protein, 213 aa, Foot-and-mouth disease virus
SGAPPTDLQKMVMGNTKPVELILDGKTVAICCATGVFGTAYLVPRHLFAEKYDKIMLDGRTMTDSDYRVFEFEIKVKGQDMLSDAALMVLHRGNRVRDITKHFRDTARMKKGTPIVGVINNADVGRLIFSGEALTYKDIVVCMDGDTMPGLFAYKAATKAGYCGGAVLAKDGADTFIVGTHSAGGNGVGYCSCVSRSMLQKMKAHIDPEPHHE

SEQ ID NO: 19 - DNA, 59 bp, Autographa californica multiple nucleopolyhedrovirus
  source 1..59: mol_type = other DNA
caaataaataagtattttactgttttcgtaacagttttgtaataaaaaaacctataaat

SEQ ID NO: 20 - DNA, 329 bp, Autographa californica multiple nucleopolyhedrovirus
  source 1..329: mol_type = other DNA
gtcttgtaaggcagtttgatttctttgctctctctccacaccagcggcaccaacgcgttggtatctttaggccaataaacaaattttttgtgtttggaattagtctttttcacgcttgatattatgttattgcaagcgctctgaataggtatacgagtgcgaaagccgttttcgtcgtacaaatcgaaatattgttgtgccagcgaataattaggaacaatataagaatttaaaattttatacaacaaatcttggctaaaatttattgaataagagatttctttctcaatcataaaattgccgtggtccatatttataacggcaacaat

SEQ ID NO: 21 - DNA, 110 bp, Autographa californica multiple nucleopolyhedrovirus
  source 1..110: mol_type = other DNA
gacctttaattcaacccaacacaatatattatagttaaataagaattattatcaaatcatttgtatattaattaaaatactatactgtaaattacattttatttacaatc

SEQ ID NO: 22 - DNA, 54 bp, Foot-and-mouth disease virus
  source 1..54: mol_type = genomic DNA
ctgctgaaccttgatctgctcaagttagcgggagacgttgagtccaaccctggc

SEQ ID NO: 23 - DNA, 54 bp, Foot-and-mouth disease virus
  source 1..54: mol_type = genomic DNA
tccttaaactttgacctgctcaagttggcaggagacgtggagtccaaccctggt

SEQ ID NO: 24 - DNA, 160 bp, Autographa californica multiple nucleopolyhedrovirus
  source 1..160: mol_type = other DNA
ctgttttcgtaacagttttgtaataaaaaaacctataaatctgttttcgtaacagttttgtaataaaaaaacctataaatctgttttcgtaacagttttgtaataaaaaaacctataaatctgttttcgtaacagttttgtaataaaaaaacctataaat